European Patent Application EP 4 553 147 A1, published May 14, 2025. Title: GENETIC ENGINEERING BACTERIUM FOR DE NOVO SYNTHESIS OF CIS,CIS-MUCONIC ACID BY TAKING GLUCOSE AS SUBSTRATE AND APPLICATIONS THEREOF. Applicant: Beijing University of Chemical Technology. Application US. The sequence listing filed with the application follows.

SEQUENCE LISTING (85 sequences)

SEQ ID NO: 1 - DNA, 1032 bp, Corynebacterium glutamicum
  source 1..1032: mol_type = genomic DNA
ctttttccagagctttttggaacagcttgccggtgacaccgtcaatatttccactgatgtacgtacgcccgtccacgtggcggaaagtcaaggtgccatcactcccctttggcccacgcttctttcctgtgaaggttggatccagttccttgatccagcgagtaatcagccctgcaagtgcggaggcttccatcagtgcctggccagcaatgcgcggtgtcagcttttcggcaatgcgatggtccaactcatcccacaactccggtttagcctgcttgactgcctgcataatgcgggccaggtacggaatccgaacgtggaagtgagtttctaccaccactcttaaaatgggcagcttcattaaagcccacatggcgttaatagcctggttgataaaatgcttggattcccccgtgacggttttcaactccatgacaagagtgctagcgtccgcctctgggtttgagatcagcaaagtccagcgctggatctccatttgcgccatggtgaagttgatgtgactctctggattatttgggtcctgatggctgaagtatgacatttccatgccccctaatggtttaaatttcccctttttaactcattagcacccaccctaaccacacaaatcaaaacaaacaagtgttctaacgaatatttgttctaattcttgaaaataaagataccgctctaccgaaactgcaggtagagcggttagaacctcaactatcccttgaggtaatactccagagcattggggtgttttgccagtggagtgatcttgacattcatgtatttgaacatcggaaagccactaagaattgcatgcagctcgtcgtggtcatcgacatcgaaaatggagtagtttgcatactcgccgacgactcgccagattgctttcatgattccacgggattgcaggtctccggagtaggccttttccttagcctggaaatctgccatcacatcggcgtccatggaatcagggaagacgacgtccatgcgtgctagaaacagcatcgataattctcc

SEQ ID NO: 2 - DNA, 1033 bp, Corynebacterium glutamicum
  source 1..1033: mol_type = genomic DNA
tttttctatggctttctggttaagtgggaaaagtcccgccacaagatgtggtcgggacttcaatgctagctaggtagaaaaactagtcttccttatccaggacgaatgggtagtgaacgtggttaccatcctcgccagtctcagggtgcaggaccagttctggcttcacagcggttgcaacgtcgttttcgacccactcgccaccctcgaagtaaagctgggtggtgatggtgcggtagcccgggtgggaaacgcgcaagtggaggtgggctgggcgccatgggtgcccaccgtaagactcaatgaaccaaccggttgggccatcatgagggatctggtaaggcgcaggctgcagggtcttgatcttgtagcggccttcctcatcggtaacgatggtgccacgcaggttccactctgggattccaggcgcgaactgggagtagtatccgtcctcatctgcgtgccagagctcaacttctgctccatcaagaccgttgccgtcgaggtcagtaacctgcccctcgaagatcagtggggtgcatgcgcggtccttgtcacgcattggcatttcagcatcccaagggagcttcggagagttctctacgtaataagggccttcgatggaacccttggttccggtgtagtcgtggcggttgtagttgatctcttcgatctcatgctcaacgaaaacgtccaaccacagtggccactcgccgtattctccaacgtcgatcatccactgcttgagcactgcgtactcttcgtaggtgacttcgtgcttgtgagcaacctgggcgatcgccgcgagcagatctacgtagatcgcgtttgcgcgttccttggaggtatcggaggaaacgcggtttgccttgaacttgtcagttgccttgttgcccgaatcgtgggctgttggatcaacgatctgttcagctgaagtcatgtcatactcctagagactttgggggtgaagtagggggtgcgagtcggatcactgcctagcggaaaaatctttgtgatcggctgaactcgataa

SEQ ID NO: 3 - DNA, 34 bp, synthetic construct
  source 1..34: mol_type = other DNA
ctagactttttccagagctttttggaacagcttg

SEQ ID NO: 4 - DNA, 48 bp, synthetic construct
  source 1..48: mol_type = other DNA
ccagaaagccatagaaaaaggagaattatcgatgctgtttctagcacg

SEQ ID NO: 5 - DNA, 31 bp, synthetic construct
  source 1..31: mol_type = other DNA
tttttctatggctttctggttaagtgggaaa

SEQ ID NO: 6 - DNA, 32 bp, synthetic construct
  source 1..32: mol_type = other DNA
ttatcgagttcagccgatcacaaagatttttc

SEQ ID NO: 7 - DNA, 35 bp, synthetic construct
  source 1..35: mol_type = other DNA
atcggctgaactcgataaaagcttggcactggccg

SEQ ID NO: 8 - DNA, 41 bp, synthetic construct
  source 1..41: mol_type = other DNA
caaaaagctctggaaaaagtctagaggatccccgggtaccg

SEQ ID NO: 9 - DNA, 23 bp, synthetic construct
  source 1..23: mol_type = other DNA
ctcaagcgtttgcgaaagaaacg

SEQ ID NO: 10 - DNA, 26 bp, synthetic construct
  source 1..26: mol_type = other DNA
gagtcagtgaacaggtaccatttgcc

SEQ ID NO: 11 - DNA, 1003 bp, Corynebacterium glutamicum
  source 1..1003: mol_type = genomic DNA
gctcaccgcgattttagagtggcgaaactctcattctttaccgttagcaaccctatggggtctcatcagctgcgccttaccttttgcggggccacttttctggattgttataagctactttaagaatagaaaaaaataaaagaatcaaagcgaagtgctatttacttgattcacccgttgataaatatttattcatatattgaagttctcggcatacattccccataaagctcataaactctgtgtcgtgacctctcagattattatgatgagttttcccttttccacgtaattgaattagcacgaagggcgattcccaaatgaccaatgggtcggatcgcctttttgctcatgctcagctcactggcgtacagcgcacagttacatttcgaccagatagcgcactggatgcactgtcgtgattacttacttctcagctatagacatactttcgctacttattctcagcgtcattatgctcatctgcagtgcgccagtcttattagtcatctttcgcagcaacagtcctgacgacctcatcgcagcactcatcctgacagcgttgttgggttttctcgctgtcaattttgtactccccacactcgcagacatcggctgcacgctgtgcgagctttaaaccagtaccccaaccagaaagtgactacgacatgagcgcaaaatcccctaccccacagcctccgtacgaaataccatcattccggaaaagacgcctaatcactaccggattattaacaatcacaacattgtggttcatctacttttatgtggatctagtaagcgccactacgctacttacgctgccggtgattatcgctgcaccattgatcatggtctacatctggtaccacgaattcacatactatgctcgtgtccgcaaaaacaataagctttacaaggctctctatgggcacctccaaaaccatcaacatcctgaaaatacggatactccacccatgtaaatagtcactaagatttagtcaca

SEQ ID NO: 12 - DNA, 1024 bp, Corynebacterium glutamicum
  source 1..1024: mol_type = genomic DNA
tccgagagccgagtaccgcttaagtctcaggcataaatcaagaactcagagacgatccggcaggacgaatgacatccacaggttcaggctgatccgtcacctcgatcacatattgaacctctgagtccgaaccatccgggaaagtcacttctgtacgaaaccacagttgaccggttcgatcatcaggcgccgtgaaggtgagatcgccagtcttctcatctatgagaatgattgcacccatcaactccgcattctcaattgagccgtaacgatctcggaccaccttcgatccctgtgggaccccaccaaccgctcctgtaccaccatccgtcaccctcaatgggatcttgacagtctgaccattgcggactttaggataacccgtgctttcaatgccgtagtaaatactgtcagccacataaaccactgaatggggtgtcactctatcaaatgacccatcagggtagaccaccttgacagtcactcgatctgtataagatcgtttcatttcaccaggggtgtagctgatccccgaagccccaagagtatgtcgaatctcccctgtatttgggtccaatcgagaagcgagcagaccatcatcaataataattgaaaacgaatcaccctcaagtaaaaatcgagtctcctctggtaattcagcaaggttttcaacagactgttcaaccgacttgggaaagactccactagaaccgagacgcgtttctaaggattcataccgtggttcatactgagcagccatagacacattttcatatgcaatcgcaacacccgtgccatttaccgttgctccgaacaacagtgaacatgacagtgcagcggtaaccaacgtgcgtgaacgtaccaacatacttctacaccactttctaaattagagatactctatgccacctcacagtataggtacaggatgtgtggcgttccctgccctcatggacggggttgctgcgtaccaactgccctacacattgcgagagccggataacgcttaagtctcaagcagaga

SEQ ID NO: 13 - DNA, 26 bp, synthetic construct
  source 1..26: mol_type = other DNA
gtcgctcaccgcgattttagagtggc

SEQ ID NO: 14 - DNA, 37 bp, synthetic construct
  source 1..37: mol_type = other DNA
gatgtgactaaatcttagtgactatttacatgggtgg

SEQ ID NO: 15 - DNA, 38 bp, synthetic construct
  source 1..38: mol_type = other DNA
gtcactaagatttagtcacatccgagagccgagtaccg

SEQ ID NO: 16 - DNA, 28 bp, synthetic construct
  source 1..28: mol_type = other DNA
tctctgcttgagacttaagcgttatccg

SEQ ID NO: 17 - DNA, 38 bp, synthetic construct
  source 1..38: mol_type = other DNA
cttaagtctcaagcagagagacctgcaggcatgcaagc

SEQ ID NO: 18 - DNA, 39 bp, synthetic construct
  source 1..39: mol_type = other DNA
taaaatcgcggtgagcgactctagaggatccccgggtac

SEQ ID NO: 19 - DNA, 1000 bp, Corynebacterium glutamicum
  source 1..1000: mol_type = genomic DNA
aacgttgacggtgatgccatcgatgctggttgcagccctgctcactgctgagtgagtgacagcagccaactcgcgcagcgttgcccactccgcgtgccagctgccggtgccgcgctgcaaacggcagtcgagggcgtcgaaaagcgttgcaagaaggccaggtgcccggcgcgcgtaaccgtcgcacgcaatcgcagcggccggattggctttgtggggcatcgcggagctgccgccgggggatttctcccgcaactcgccgacctcggtttgtgagtaaaacaccacgtcaccagcaattttgcgtaccacaccagcggccgttgccagcgccgacgcgatcgcagtgatcggcgtgcgatcggaatgccacacccactgcggatcaaaaaggcccaactcctcggccagcttcgcctgaatctcgaagccacgcgggtgcaccgccgtcatatttccgctggcaccgccatacgacaccggaaactccagcgcctccagggcgcgtgccgcattgtccaccgcaaccagccagccgccggtcagcgcgccgaacgtcgtcggcgtcgcgatctgccccaacgtgcgccccatgatcggggttgctttatgctccgcggtgagctcggccaaatctcgcgcaagctttttaagcttgtcgacgacctcccccaccccttccttcatgcacagcattaacgcagaatcaatgatgtcctggctcgttgcgccaatgtggatgcctgccggattgatggccttgaggtcagtgaccagcggaatgagcggattaccgccctcggctgcgcgacgggaaagctcctccacatccaactgataagaatcaatggtggccttcgccattgctgcgtgctcgggggcagctgcaaccgccaaagcggcctccacgacaagaagattctttaggaaagtctcgtcggaaaggctgctgaggtgttctccactaccagcaaggtcggagtataaagatcgggtcaat

SEQ ID NO: 20 - DNA, 1000 bp, Corynebacterium glutamicum
  source 1..1000: mol_type = genomic DNA
gcgagacctttctgcgtctagtgatatagatctcaaagtagggatgattgaggccgttgacaagtagttcgcggggcgaacatgtcagatcgcgcgcgaacattcgccaccagcgcaaaccccgaaggtcaggggttaactaggggtgtgcataagggtttagtcatccaatacctcgagtgaactgcggagcttttcaaaagtcttctccatccgtgcttccagagtctgcccccactgccccgtgggcatctcttgcgccaacggtccgacaggttcggttaccactgtgcgattgcacggcccaatccaggcgacccgacccatggaatcaatcgccgcctggatgcgcccatcagtcttcatattgtgatgatgcgcgcagaggcactgcaagttccaggccacagtcaacccaccctcaccgaacgggatcacgtgatcgatctggcagttgtcggcagacaccgtgcagcccggatgcctacaggtgccgtcccgccccatcacataaaggcgtagctcgggacttggggtgtagccattttccacacgagtggcgatcgtatccaggtcaatgaccttcgaggcagtcttacccagcttccgggactcctcttgactcaggaatcccacccccggaatccaggacacgccacccaccaggggcgtgtataccgcgctgacgattttcactttggtccgccccgccaggaaggtgaccagggcccgcgcgaggtcctcgcccttctgtttcactttttccagagctttttggaacagcttgccggtgacaccgtcaatatttccactgatgtacgtacgcccgtccacgtggcggaaagtcaaggtgccatcactcccctttggcccacgcttctttcctgtgaaggttggatccagttccttgatccagcgagtaatcagccctgcaagtgcggaggcttccatcagtgcctggccagcaatgcgcggtgtcagcttttcggcaatgcgatgg

SEQ ID NO: 21 - DNA, 21 bp, synthetic construct
  source 1..21: mol_type = other DNA
aacgttgacggtgatgccatc

SEQ ID NO: 22 - DNA, 29 bp, synthetic construct
  source 1..29: mol_type = other DNA
attgacccgatctttatactccgaccttg

SEQ ID NO: 23 - DNA, 44 bp, synthetic construct
  source 1..44: mol_type = other DNA
gagtataaagatcgggtcaatgcgagacctttctgcgtctagtg

SEQ ID NO: 24 - DNA, 22 bp, synthetic construct
  source 1..22: mol_type = other DNA
ccatcgcattgccgaaaagctg

SEQ ID NO: 25 - DNA, 35 bp, synthetic construct
  source 1..35: mol_type = other DNA
ttcggcaatgcgatgggacctgcaggcatgcaagc

SEQ ID NO: 26 - DNA, 29 bp, synthetic construct
  source 1..29: mol_type = other DNA
atcaccgtcaacgttgactctagaggatc

SEQ ID NO: 27 - DNA, 1000 bp, Corynebacterium glutamicum
  source 1..1000: mol_type = genomic DNA
caacagaggtgccgttgtcaaagaattcctccccctttaggcgtgagaccagcatgtccagatcctcacggactggaacgatcactgctacatcagcaagacccaaggttgctgcgcgtggacctgcacctgctgagttccaggtgttcatggccacatggtggtgatatccacctgcggaggcaaacagtgcattggggattgatgtggtggcatcaaaaccaatcttgtccacatagaattgacgggctcgctcgacgttgcctacctgaaggtgaacgtgtccgatgctcgcagggagaatagcggtgttgttcaaaacggtttcgctgagatgactctgaaggtactggtttggatccaagtagatggtgtccatgcggacatcgccgttgtctgcatacttccatgcacttcgagggcggtcaacatagagctcaatgccgtttccctcaggatcggtgaagtaaaaagcttcagagactaggtgatctgaagaacccacaaaacgtgagcgtgattcttgcgctgcgcggtaaacggtggcagccaagctctcttgggtatcgaagaggaaagcggtgtgataaaggccagcttgacgaggatctaccgcaggaagacctggggtagaaatcaggcgaagcagtggggtgccattgcgaccgagtacacggtgaacttcttttccgtgaactttttcttccattggttcaacgctaaggattgaagagtagtaactagtcataccctctaggtcgccgacgcgaaggctaactgcatccatgaaggtgtcgctattgatgctctgctcaagaagtgccatggtgtttcatcctttaagtgttggtggctgttttgctgttgaacaccattgttcaccaatttactttccgtgtcaagtaaattcttaaatgaggcggatttcccctgccctagccacgaaaaatgcgctgacaccacgtacagtgtcaacgcattttttgaaagatttaagcga

SEQ ID NO: 28 - DNA, 1001 bp, Corynebacterium glutamicum
  source 1..1001: mol_type = genomic DNA
gcccataagcctagtacgtcattccccctcaagccacaggtactaccattaattctcgatgaatcttgcgacccagagtgtgaacagacaatgttctacgcctctgacgtgcttaaatcagaaaaaaccgggcacccacaaaacaattcgggcactcggtttttctaccaaaaacatctcagccaggtcaggcctatggttgaaacctatcgcgttgagggcgtttctccatcaatgccctcccctgctttcggcaagggttttccatccggcgaagctacagcatctgctgcaacagacgctgcgaaagtcggatctacctcttcgggagtttccctacccttcttcaacaggaagaacacgatgatcgcgccggcaaacactactgcggagacgatggtgttgattcggatgccgccaataagcgtggcttcatcaacgcgcatttgttcaatccagaaacggcccaaggtataaccagctacgtagagtgcaaatactcggccatgtcccagcttgaatcgcttgtcagcccacatcaacaaagcgaagatcagtaggttccacaacagttcatagaggaatgttggatgaacagtagccattacttcaccggtggatgttcctgtcaccggtgcgaattttccattttcatctacccgatagtagatttccaaagcccatggaacggtagtttctgcaccgtagagctcctggttaaaccagttgcccagacgaccaattccctgcgccaggataactgcaggtgccacggcatctgcgaaaggtgcaagaggaagctttttgtaccggaagaatacggccactgccaggccaccgaggatcactgcaccccagatgcccagaccaccgttggtgattttgaaggcgtcgacggggttacaggtatcgcagaagtacttttggttgtcggtaatgacgtgataaatgcgtccaccgatgattccggcaggaactgccacgatcgctgcatcaaggac

SEQ ID NO: 29 - DNA, 33 bp, synthetic construct
  source 1..33: mol_type = other DNA
ctctagagtccaacagaggtgccgttgtcaaag

SEQ ID NO: 30 - DNA, 35 bp, synthetic construct
  source 1..35: mol_type = other DNA
ggctcgcttaaatctttcaaaaaatgcgttgacac

SEQ ID NO: 31 - DNA, 40 bp, synthetic construct
  source 1..40: mol_type = other DNA
gaaagatttaagcgagcccataagcctagtacgtcattcc

SEQ ID NO: 32 - DNA, 27 bp, synthetic construct
  source 1..27: mol_type = other DNA
caggtcgtccttgatgcagcgatcgtg

SEQ ID NO: 33 - DNA, 29 bp, synthetic construct
  source 1..29: mol_type = other DNA
catcaaggacgacctgcaggcatgcaagc

SEQ ID NO: 34 - DNA, 31 bp, synthetic construct
  source 1..31: mol_type = other DNA
ctctgttggactctagaggatccccgggtac

SEQ ID NO: 35 - DNA, 858 bp, Corynebacterium glutamicum
  source 1..858: mol_type = genomic DNA
atgacttcagctgaacagatcgttgatccaacagcccacgattcgggcaacaaggcaactgacaagttcaaggcaaaccgcgtttcctccgatacctccaaggaacgcgcaaacgcgatctacgtagatctgctcgcggcgatcgcccaggttgctcacaagcacgaagtcacctacgaagagtacgcagtgctcaagcagtggatgatcgacgttggagaatacggcgagtggccactgtggttggacgttttcgttgagcatgagatcgaagagatcaactacaaccgccacgactacaccggaaccaagggttccatcgaaggcccttattacgtagagaactctccgaagctcccttgggatgctgaaatgccaatgcgtgacaaggaccgcgcatgcaccccactgatcttcgaggggcaggttactgacctcgacggcaacggtcttgatggagcagaagttgagctctggcacgcagatgaggacggatactactcccagttcgcgcctggaatcccagagtggaacctgcgtggcaccatcgttaccgatgaggaaggccgctacaagatcaagaccctgcagcctgcgccttaccagatccctcatgatggcccaaccggttggttcattgagtcttacggtgggcacccatggcgcccagcccacctccacttgcgcgtttcccacccgggctaccgcaccatcaccacccagctttacttcgagggtggcgagtgggtcgaaaacgacgttgcaaccgctgtgaagccagaactggtcctgcaccctgagactggcgaggatggtaaccacgttcactacccattcgtcctggataaggaagactag

SEQ ID NO: 36 - DNA, 15 bp, synthetic construct
  source 1..15: mol_type = other DNA
aaggaggatatacat

SEQ ID NO: 37 - DNA, 1509 bp, Kleber pneumoniae
  source 1..1509: mol_type = genomic DNA
atgaccgcaccgattcaggatctgcgcgacgccatcgcgctgctgcaacagcatgacaatcagtatctcgaaaccgatcatccggttgaccctaacgccgagctggccggtgtttatcgccatatcggcgcgggcggcaccgtgaagcgccccacccgcatcgggccggcgatgatgtttaacaatattaagggttatccacactcgcgcattctggtgggtatgcacgccagccgccagcgggccgcgctgctgctgggctgcgaagcctcgcagctggcccttgaagtgggtaaggcggtgaaaaaaccggtcgcgccggtggtcgtcccggccagcagcgccccctgccaggaacagatctttctggccgacgatccggattttgatttgcgcaccctgcttccggcgcccaccaacacccctatcgacgccggccccttcttctgcctgggcctggcgctggccagcgatcccgtcgacgcctcgctgaccgacgtcaccatccaccgcttgtgcgtccagggccgggatgagctgtcgatgtttcttgccgccggccgccatatcgaagtgtttcgccaaaaggccgaggccgccggcaaaccgctgccgataaccatcaatatgggtctcgatccggccatctatattggcgcctgcttcgaagcccctaccacgccgttcggctataatgagctgggcgtcgccggcgcgctgcgtcaacgtccggtggagctggttcagggcgtcagcgtcccggagaaagccatcgcccgcgccgagatcgttatcgaaggtgagctgttgcctggcgtgcgcgtcagagaggatcagcacaccaatagcggccacgcgatgccggaatttcctggctactgcggcggcgctaatccgtcgctgccggtaatcaaagtcaaagcagtgaccatgcgaaacaatgcgattctgcagaccctggtgggaccgggggaagagcataccaccctcgccggcctgccaacggaagccagtatctggaatgccgtcgaggccgccattccgggctttttacaaaatgtctacgcccacaccgcgggtggcggtaagttcctcgggatcctgcaggtgaaaaaacgtcaacccgccgatgaaggccggcaggggcaggccgcgctgctggcgctggcgacctattccgagctaaaaaatattattctggttgatgaagatgtcgacatctttgacagcgacgatatcctgtgggcgatgaccacccgcatgcagggggacgtcagcattacgacaatccccggcattcgcggtcaccagctggatccgtcccagacgccggaatacagcccgtcgatccgtggaaatggcatcagctgcaagaccatttttgactgcacggtcccctgggcgctgaaatcgcactttgagcgcgcgccgtttgccgacgtcgatccgcgtccgtttgcaccggagtatttcgcccggctggaaaaaaaccagggtagcgcaaaataa

SEQ ID NO: 38 - DNA, 594 bp, Kleber pneumoniae
  source 1..594: mol_type = genomic DNA
atgaaactgattattgggatgacgggggccaccggggcaccgcttggggtggcattgctgcaggcgctgcgcgatatgccggaggtggaaacccatctggtgatgtcgaaatgggccaaaaccaccatcgagctggaaacgccctggacggcgcgcgaagtggccgcgctggcggacttttcccacagcccggcagaccaggccgccaccatctcatccggttcatttcgtaccgacggcatgatcgttattccctgcagtatgaaaacgcttgcaggcattcgcgcgggttatgccgaagggctggtgggccgcgcggcggacgtggtgctcaaagaggggcgcaagctggtgttggtcccgcgggaaatgccgctcagcacgatccatctggagaacatgctggcgctgtcccgcatgggcgtggcgatggtcccgccgatgccagcttactacaaccacccggagacggttgacgatatcaccaatcatatcgtcacccgggtgctggatcagtttggcctcgactatcacaaagcgcgccgctggaacggcttgcgcacggcagaacaatttgcacaggagatcgaataa

SEQ ID NO: 39 - DNA, 237 bp, Kleber pneumoniae
  source 1..237: mol_type = genomic DNA
atgatttgtccacgttgcgccgatgaaaagattgaagtcatggcgacctcgccggtgaaaggggtctggaccgtgtatcagtgccagcactgtctttacacctggcgagataccgagccgctgcgccgcaccagccgcgaacactatccggaagcgttccgcatgacgcagaaagatatcgatgaggcgccgcaggtgccgcacgtaccgccgctattgccggaagataagcgttaa

SEQ ID NO: 40 - DNA, 31 bp, synthetic construct
  source 1..31: mol_type = other DNA
catatgacttcagctgaacagatcgttgatc

SEQ ID NO: 41 - DNA, 28 bp, synthetic construct
  source 1..28: mol_type = other DNA
ctagtcttccttatccaggacgaatggg

SEQ ID NO: 42 - DNA, 56 bp, synthetic construct
  source 1..56: mol_type = other DNA
cctggataaggaagactagaaggaggatatacatatgaccgcaccgattcaggatc

SEQ ID NO: 43 - DNA, 63 bp, synthetic construct
  source 1..63: mol_type = other DNA
atcccaataatcagtttcatatgtatatcctccttttattttgcgctaccctggtttttttcc

SEQ ID NO: 44 - DNA, 30 bp, synthetic construct
  source 1..30: mol_type = other DNA
catatgaaactgattattgggatgacgggg

SEQ ID NO: 45 - DNA, 28 bp, synthetic construct
  source 1..28: mol_type = other DNA
ttattcgatctcctgtgcaaattgttct

SEQ ID NO: 46 - DNA, 53 bp, synthetic construct
  source 1..53: mol_type = other DNA
gcacaggagatcgaataaaaggaggatatacatatgatttgtccacgttgcgc

SEQ ID NO: 47 - DNA, 28 bp, synthetic construct
  source 1..28: mol_type = other DNA
gattaacgcttatcttccggcaatagcg

SEQ ID NO: 48 - DNA, 40 bp, synthetic construct
  source 1..40: mol_type = other DNA
cggaagataagcgttaatctagagtcgacctgcaggcatg

SEQ ID NO: 49 - DNA, 57 bp, synthetic construct
  source 1..57: mol_type = other DNA
gttcagctgaagtcatatgtatatcctccttgagctcgaattcttctgtttcctgtg

SEQ ID NO: 50 - DNA, 1857 bp, Corynebacterium glutamicum
  source 1..1857: mol_type = genomic DNA
atgcgtacatccattgccactgtttgtttgtccggaactcttgctgaaaagctgcgcgcagctgcagatgctggatttgatggtgtggaaatcttcgagcaggacttggtggtttccccgcattcggcagagcagattcgtcagcgggctcaggatttgggattaaccctggatctgttccagccgtttcgagatttcgaaggtgtggaagaagagcagtttctgaagaatctgcaccgcttggaagagaagttcaagctgatgaacaggcttggcattgagatgatcttgttgtgttccaatgtgggcaccgcgaccatcaatgatgatgaccttttcgtggagcagttgcatcgtgcagcagatttggctgagaagtacaacgtcaagattgcttatgaagcgttggcgtggggcaagtttgtcaatgattttgagcatgcgcatgcacttgtggagaaggtgaatcacaaggcgctgggaacctgcttggatacgttccatattctttcccgtggttgggaaaccgacgaggtggagaacatccctgcggagaagatcttctttgttcagttagcggatgcgccgaagctgagcatggacattttgtcctggtcgcgtcaccaccgtgttttccctggtgaaggcgatttcgatctggtgaaattcatggttcatctggccaagacgggttatgatggcccgatttctttggagatcttcaacgattccttccgcaaggccgaggttggtcgcaccgcgattgatgggttgcgttctttgcgttggttggaagatcagacctggcatgcgctaaatgctgaggatcgtccaagcgctcttgaactgcgtgcacttcctgaggtcgcggaacctgagggtgttgatttcattgagatcgccactggacgtttgggtgagaccattcgggttcttcatcaattgggtttccgcttgggtggtcatcactgcagtaagcaggattaccaggtatggacccagggcgatgtgcgcattgtggtgtgtgatcgtggggtcaccggggctccaaccacgatctctgcgatgggctttgacacccccgatccagaagctgctcatgcccgtgcggaattgctgcgggctcagacaattgatcgtccccacatcgagggcgaagttgacctaaaaggtgtgtacgcaccggatggggtggagctgtttttcgcggggccgagccccgatggaatgcccgagtggctgccggaattcggcgtcgaaaagcaagaagctggtctcattgaagccatcgaccacgtcaatttcgcccagccgtggcaacattttgatgaggcagtgctgttttacaccgcgctgatggcgttggagactgtgcgtgaggatgagttcccgagcccaattggtttggtgcgcaatcaggtgatgcgttcgccgaatgatgcggtgcggttgctgctcagcgtggcgccggaggacggtgagcagggagatttcctcaacgcggcctacccggagcacattgcgttggccacggcggacatcgtggcggtggctgaacgtgcgcgcaaacgaggcctggatttcttgcccgtcccagagaattactacgacgatgtgcaggcgcgttttgatttgccgcaggaattcttggacacactcaaggaaaaccacctgctttacgaccgcgacgagaacggcgaattcctccacttttacacccgcacgttgggcacgctgttcttcgaagtggtggaacgccgcggcggttttgcaggttggggcgaaacaaacgctccggtgcggttggcggcgcagtatcgtgaggtgcgggacctcgagcggggaatcccaaactag

SEQ ID NO: 51 - DNA, 1098 bp, Corynebacterium glutamicum
  source 1..1098: mol_type = genomic DNA
atgagcgcagtgcagattttcaacaccgtccacgtcaatggatcttccccctatgatgtccacattggttccggcctcaacgagctcattgttcagcgcgcagcggaatcaggcgcggagcaggtagcgattttgcaccagcccagcatggatgacattgcatccgagttggatgcagcactagtcgctgctggtttgaaggtcctgcaccttaatgttcccgatgcggaaaacggcaagtccttggaagtagcggggcagtgctgggatgaattgggtggcgcagcattcggccgccgcgatatcgtcatcggacttggtggcggtgctgccacagatctcgcgggattcgtcgctgctgcatggatgcgtggcgtgcgcgtcattcaggttccaaccaccttgttggccatggtggacgctgcggtgggcggcaagactggcatcaataccgccgcaggcaagaaccttgtgggcgcgttccacgagcctgacgcagtattcattgacaccgatcgcctagccaccctgcctgacgcggaaatcatcgcgggatccgccgaaatcatcaaaactggtttcatcgccgacccagaaatcctgcgcctttacgaaactgatcccgcagcctgcctgaagaaagaagtcgaaggctcccacctacctgaactgatttggcgctccgtcaccgtcaagggctccgtggtcggccaagacctcaaagaatctagcctgcgcgaaatcctcaactacggacacacctttgcccacgccgtcgaactccgcgaaaacttccgctggcgccacggcaatgccgttgcagtgggcatgatgttcatcgccaacctctcccacaagctcgggcttatcgacgcgcccctcctcgagcgccaccgctcaatcctggcggccatcggtctgcccacttcctacgaaggcggagccttcgacgagctttacgacggtatgacccgcgacaagaaaaaccgcgacggcaacatccgcttcgtcgcactgaccgccgtgggcgaggttacccgcattgaggggccctcaaaacaagatttacagagtgcttatgaggcaatcagccactaa

SEQ ID NO: 52 - DNA, 438 bp, Corynebacterium glutamicum
  source 1..438: mol_type = genomic DNA
atgcctggaaaaattctcctcctcaacggcccaaacctgaacatgctgggcaaacgcgagcctgacatttacggacacgacaccttggaagacgtcgtcgcgctggcaaccgctgaggctgcgaagcacggccttgaggttgaggcgctgcagagcaatcacgaaggtgagctaatcgatgcgctgcacaacgctcgcggcacccacatcggttgcgtgattaaccccggcggcctgactcacacttcggtggcgcttttggatgctgtgaaggcgtctgagcttcctaccgttgaggtgcacatttccaatccgcatgcccgtgaagagttccgccaccattcttacatttccctcgccgcggtctccgttatcgctggcgctggcatccagggttaccgtttcgcggtcgatatcctggcaaatctcaaaaagtag

SEQ ID NO: 53 - DNA, 1995 bp, Corynebacterium glutamicum
  source 1..1995: mol_type = genomic DNA
atgtcctcacgtaaagagcttgccaatgctattcgtgcgctgagcatggacgcagtacagaaagccaaatccggtcacccgggggcccctatgggtatggctgacattgccgaagtcctgtggcgtgatttcctgaaacacaacccgcagaatccgtcctgggctgaccgtgaccgcttcgtgctgtccaacggccacggctccatgctgatctacagcctgctgcacctcaccggttacgatctgccgatggaagaactgaaaaacttccgtcagctgcactctaaaactccgggtcacccggaaagtggggttacaccgctgggtgtggaaaccaccaccggtccgctgggtcagggtattgccaacgcagtcggtatggcgattgcagaaaaaacgctggcggcgcagtttaaccgtccgggccacgacattgtcgaccactacacctacgccttcatgggcgacggctgcatgatggaaggcatctcccacgaagtttgctctctggcgggtacgctgaagctgggtaaactgattgcattctacgatgacaacggtatttctatcgatggtcacgttgaaggctggttcaccgacgacaccgcaatgcgtttcgaagcttacggctggcacgttattcgcgacatcgacggtcatgacgcggcatctatcaaacgcgcagtagaagaagcgcgcgcagtgactgacaaaccttccctgctgatgtgcaaaaccatcatcggtttcggttccccgaacaaagccggtacccacgactcccacggtgcgccgctgggcgacgctgaaattgccctgacccgcgaacaactgggctggaaatatgcgccgttcgaaatcccgtctgaaatctatgctcagtgggatgcgaaagaagcaggccaggcgaaagaatccgcatggaacgagaaattcgctgcttacgcgaaagcttatccgcaggaagccgctgaatttacccgccgtatgaaaggcgaaatgccgtctgacttcgacgctaaagcgaaagagttcatcgctaaactgcaggctaatccggcgaaaatcgccagccgtaaagcgtctcagaatgctatcgaagcgttcggtccgctgttgccggaattcctcggcggttctgctgacctggcgccgtctaacctgaccctgtggtctggttctaaagcaatcaacgaagatgctgcgggtaactacatccactacggtgttcgcgagttcggtatgaccgcgattgctaacggtatctccctgcacggtggcttcctgccgtacacctccaccttcctgatgttcgtggaatacgcacgtaacgccgtacgtatggctgcgctgatgaaacagcgtcaggtgatggtttacacccacgactccatcggtctgggcgaagacgggccgactcaccagccggttgagcaggtcgcttctctgcgcgtaaccccgaacatgtctacatggcgtccgtgtgaccaggttgaatccgcggtcgcgtggaaatacggtgttgagcgtcaggacggcccgaccgcactgatcctctcccgtcagaacctggcgcagcaggaacgaactgaagagcaactggcaaacatcgcgcgcggtggttatgtgctgaaagactgcgccggtcagccggaactgattttcatcgctaccggttcagaagttgaactggctgttgctgcctacgaaaaactgactgccgaaggcgtgaaagcgcgcgtggtgtccatgtcgtctaccgacgcatttgacaagcaggatgctgcttaccgtgaatccgtactgccgaaagcggttactgcacgcgttgctgtagaagcgggtattgctgactactggtacaagtatgttggcctgaacggtgctatcgtcggtatgaccaccttcggtgaatctgctccggcagagctgctgtttgaagagttcggcttcactgttgataacgttgttgcgaaagcaaaagaactgctgtaa

SEQ ID NO: 54 - DNA, 25 bp, synthetic construct
  source 1..25: mol_type = other DNA
catatgcgtacatccattgccactg

SEQ ID NO: 55 - DNA, 22 bp, synthetic construct
  source 1..22: mol_type = other DNA
ctagtttgggattccccgctcg

SEQ ID NO: 56 - DNA, 56 bp, synthetic construct
  source 1..56: mol_type = other DNA
ggggaatcccaaactagaaggaggatatacatatgagcgcagtgcagattttcaac

SEQ ID NO: 57 - DNA, 27 bp, synthetic construct
  source 1..27: mol_type = other DNA
cttttagtggctgattgcctcataagc

SEQ ID NO: 58 - DNA, 48 bp, synthetic construct
  source 1..48: mol_type = other DNA
gcaatcagccactaaaaggaggatatacatatgcctggaaaaattctc

SEQ ID NO: 59 - DNA, 62 bp, synthetic construct
  source 1..62: mol_type = other DNA
ctttacgtgaggacatatgtatatcctccttctactttttgagatttgccaggatatcgacc

SEQ ID NO: 60 - DNA, 55 bp, synthetic construct
  source 1..55: mol_type = other DNA
gcaaatctcaaaaagtagaaggaggatatacatatgtcctcacgtaaagagcttg

SEQ ID NO: 61 - DNA, 38 bp, synthetic construct
  source 1..38: mol_type = other DNA
ggggatcctctagattacagcagttcttttgctttcgc

SEQ ID NO: 62 - DNA, 25 bp, synthetic construct
  source 1..25: mol_type = other DNA
gtaatctagaggatccccgggtacc

SEQ ID NO: 63 - DNA, 49 bp, synthetic construct
  source 1..49: mol_type = other DNA
caatggatgtacgcatatgtatatcctccttgtcgacctgcaggcatgc

SEQ ID NO: 64 - DNA, 29 bp, synthetic construct
  source 1..29: mol_type = other DNA
gtgaaaccagtaacgttatacgatgtcgc

SEQ ID NO: 65 - DNA, 19 bp, synthetic construct
  source 1..19: mol_type = other DNA
ctcactgcccgctttccag

SEQ ID NO: 66 - DNA, 18 bp, synthetic construct
  source 1..18: mol_type = other DNA
cttcaccgcctggccctg

SEQ ID NO: 67 - DNA, 23 bp, synthetic construct
  source 1..23: mol_type = other DNA
cgcccggaagagagtcaattcag

SEQ ID NO: 68 - DNA, 594 bp, Escherichia coli
  source 1..594: mol_type = genomic DNA
atgaaactgatcgtcgggatgacaggggctaccggtgcgcctcttggtgtggcattactgcaagcgctgcgggagatgccgaatgtcgagactcatctggtgatgtcgaagtgggcgaaaaccaccattgaactggaaacgccttacagcgcccgcgatgttgctgccctcgctgacttcagccataacccggcggatcaggcggcgaccatctcctcaggttcctttcgtacagacggcatgatcgttattccgtgcagtatgaaaacgctcgccggtatccgcgctggttacgctgatggcctggtagggcgcgcggcggacgtcgtgcttaaagaaggccgcaaactggtgctggtgccgcgtgaaatgccgcttagcaccatccatctcgaaaatatgctcgcactttcacgcatgggcgtggcgatggtgccgccgatgcctgccttttataaccatcccgaaacggtagatgacattgtccaccacgtggtagcccgcgtgctggatcaatttggccttgaacatccctacgccaggcgctggcaaggattgccgcaggcccggaatttttctcaggagaatgaataa

SEQ ID NO: 69 - DNA, 237 bp, Escherichia coli
  source 1..237: mol_type = genomic DNA
atgatttgtccacgttgtgccgatgaacagattgaagtgatggcgaaatcgccggtgaaagatgtctggacggtatatcagtgccagcattgcctttatacctggcgcgataccgaaccgctgcgccgtaccagccgcgaacattatcccgaagcgttccgcatgacgcagaaagatattgatgacgcgccaatggtgccgagcatcccgccgctgctggcggaaggtaagcgctaa

SEQ ID NO: 70 - DNA, 28 bp, synthetic construct
  source 1..28: mol_type = other DNA
catatgaaactgatcgtcgggatgacag

SEQ ID NO: 71 - DNA, 33 bp, synthetic construct
  source 1..33: mol_type = other DNA
cttttattcattctcctgagaaaaattccgggc

SEQ ID NO: 72 - DNA, 56 bp, synthetic construct
  source 1..56: mol_type = other DNA
ttctcaggagaatgaataaaaggaggatatacatatgatttgtccacgttgtgccg

SEQ ID NO: 73 - DNA, 23 bp, synthetic construct
  source 1..23: mol_type = other DNA
gattagcgcttaccttccgccag

SEQ ID NO: 74 - DNA, 39 bp, synthetic construct
  source 1..39: mol_type = other DNA
ggaaggtaagcgctaatctagagtcgacctgcaggcatg

SEQ ID NO: 75 - DNA, 59 bp, synthetic construct
  source 1..59: mol_type = other DNA
cgacgatcagtttcatatgtatatcctccttttattttgcgctaccctggtttttttcc

SEQ ID NO: 76 - DNA, 1440 bp, Pseudomonas putida
  source 1..1440: mol_type = genomic DNA
atgagcaagattctcaccaccgccagcggtgcacctgtagccgacaaccagaactcccgctccgccggcccacgcggcccgctgctgctcgacgacttccacctgatcgagaagctcgcccatttcaaccgtgagaacatccccgagcgccgggtacacgcgaagggttcgggcgcctatggcacttttaccgtaacccgcgacatcaccggttacaccagcgccaaactgttcgagcaggttggcaagcagaccgagacatttctgcgcttctctaccgtgggtggcgaacgtggttctgcggacacagagcgagaccctcgcggatttgccgttaagttctacaccgaggaaggtaactgggacatcgtgggtaacaacacgccagtgttcttcattcgtgatccgctcaagttcccggactttatccacacccagaaacggcacccgcagtccaacctgaaaaacgcccaaatattttgggattcctggtcgcactcgcccgaggcgctgcaccaagtcaccatcctgttctctgatcgtggcattccggacggctaccgccacatgcacggctttggcagccacacctacagcctgatcaatgcccagggtgagcgcacttgggtcaaatggcacttcaagacccagcagggcatcaagaaccttgctccggcagatgccgcacgtttggcaggtactgacccggactacgcccagcgcgacctgttcgaagccattgagcgaggtgattacccacgctggactgtctgcatccaggtgatgagcgaagccgaagccgcgagccgcgacgagaacccgttcgacgtgaccaaaacctggtcacaaaaggactacccgttgatcgaagtgggcgtgcttgagcttaaccgtaacccgctcaattacttcgccgaagtcgagcaggctgccttcgggccaagcaacatggtgccgggggtcggcctgtcgccagaccgcatgctccagggtcgcgtattcgcctacgcggacgcacaccgctaccgtgtgggtaccaaccaccaacagttgccggtgaatgcgccacgctgcccggtcaacagctaccagcgcgacggctccatggccactggcagctatggcagtgcgccgaactacgaacccaacagctacgccgcggcaccgaagcagtcgccacgtcacgcagagcccgcattggccctgaatggttcggccgaccgttacgatcaccgcgaggacgctgactactacagccacgccggcgcgctgttccgcctgatgagtgatgagcagaaggccctgctgatcagcaacatcgctggaaccatggcgggtgtcagcgaaaacgtcatccaacggcagttgcagtacttcttcaaggccgacccagcctacggagaaggcatcgccaagggcctgggcatcaatctcgcctaa

SEQ ID NO: 77 - DNA, 26 bp, synthetic construct
  source 1..26: mol_type = other DNA
catatgagcaagattctcaccaccgc

SEQ ID NO: 78 - DNA, 25 bp, synthetic construct
  source 1..25: mol_type = other DNA
cttttaggcgagattgatgcccagg

SEQ ID NO: 79 - DNA, 42 bp, synthetic construct
  source 1..42: mol_type = other DNA
catcaatctcgcctaaaaggaggatatacatatgaccgcacc

SEQ ID NO: 80 - DNA, 59 bp, synthetic construct
  source 1..59: mol_type = other DNA
ggtgagaatcttgctcatatgtatatcctccttgagctcgaattcttctgtttcctgtg

SEQ ID NO: 81 - DNA, 1053 bp, Corynebacterium glutamicum
  source 1..1053: mol_type = genomic DNA
atgaattatcagaacgacgatttacgcatcaaagaaatcaaagagttacttcctcctgtcgcattgctggaaaaattccccgctactgaaaatgccgcgaatacggttgcccatgcccgaaaagcgatccataagatcctgaaaggtaatgatgatcgcctgttggttgtgattggcccatgctcaattcatgatcctgtcgcggcaaaagagtatgccactcgcttgctggcgctgcgtgaagagctgaaagatgagctggaaatcgtaatgcgcgtctattttgaaaagccgcgtaccacggtgggctggaaagggctgattaacgatccgcatatggataatagcttccagatcaacgacggtctgcgtatagcccgtaaattgctgcttgatattaacgacagcggtctgccagcggcaggtgagtttctcaatatgatcaccccacaatatctcgctgacctgatgagctggggcgcaattggcgcacgtaccaccgaatcgcaggtgcaccgcgaactggcatcagggctttcttgtccggtcggcttcaaaaatggcaccgacggtacgattaaagtggctatcgatgccattaatgccgccggtgcgccgcactgcttcctgtccgtaacgaaatgggggcattcggcgattgtgaataccagcggtaacggcgattgccatatcattctgcgcggcggtaaagagcctaactacagcgcgaagcacgttgctgaagtgaaagaagggctgaacaaagcaggcctgccagcacaggtgatgatcgatttcagccatgctaactcgtccaaacaattcaaaaagcagatggatgtttgtgctgacgtttgccagcagattgccggtggcgaaaaggccattattggcgtgatggtggaaagccatctggtggaaggcaatcagagcctcgagagcggggagccgctggcctacggtaagagcatcaccgatgcctgcatcggctgggaagataccgatgctctgttacgtcaactggcgaatgcagtaaaagcgcgtcgcgggtaa

SEQ ID NO: 82 - DNA, 37 bp, synthetic construct
  source 1..37: mol_type = other DNA
catatgaattatcagaacgacgatttacgcatcaaag

SEQ ID NO: 83 - DNA, 21 bp, synthetic construct
  source 1..21: mol_type = other DNA
cttttacccgcgacgcgcttt

SEQ ID NO: 84 - DNA, 43 bp, synthetic construct
  source 1..43: mol_type = other DNA
cgtcgcgggtaaaaggaggatatacatatgtcctcacgtaaag

SEQ ID NO: 85 - DNA, 64 bp, synthetic construct
  source 1..64: mol_type = other DNA
gtcgttctgataattcatatgtatatcctccttctactttttgagatttgccaggatatcgacc